European Patent Application EP 4 759 373 A2, published June 17, 2026. Title: ANTI-uPAR ANTIBODIES AND USES THEREOF. Applicant: MEMORIAL SLOAN-KETTERING CANCER CENTER. Application EP. The sequence listing filed with the application follows.

SEQUENCE LISTING (116 sequences)

SEQ ID NO: 1 - protein, 8 aa, synthetic construct
  REGION 1..8: note = Description of sequence: antibody component
GFTFSDDY

SEQ ID NO: 2 - protein, 8 aa, synthetic construct
  REGION 1..8: note = Description of sequence: antibody component
ISGSGGST

SEQ ID NO: 3 - protein, 21 aa, synthetic construct
  REGION 1..21: note = Description of sequence: antibody component
ATGVPYCSTTRCPPYYYTMDV

SEQ ID NO: 4 - protein, 7 aa, synthetic construct
  REGION 1..7: note = Description of sequence: antibody component
QSVDSTA

SEQ ID NO: 5 - skipped

SEQ ID NO: 6 - protein, 9 aa, synthetic construct
  REGION 1..9: note = Description of sequence: antibody component
QQDGEYPLT

SEQ ID NO: 7 - protein, 128 aa, synthetic construct
  REGION 1..128: note = Description of sequence: antibody component
EVQLLESGGGLVQPGGSLRLSCAASGFTFSDDYMSWVRQAPGKGLEWVSVISGSGGSTDYADSVKGRFTISRDNSKNTLYLQMNSLRAEDTAVYYCATGVPYCSTTRCPPYYYTMDVWGQGTTVTVSS

SEQ ID NO: 8 - protein, 108 aa, synthetic construct
  REGION 1..108: note = Description of sequence: antibody component
EIVLTQSPGTLSLSPGERATLSCRASQSVDSTALAWYQQKPGQAPRLLIYAASSRATGIPDRFSGSGSGTDFTLTISRLEPEDFAVYYCQQDGEYPLTFGQGTKVEIK

SEQ ID NO: 9 - protein, 255 aa, synthetic construct
  REGION 1..255: note = Description of sequence: antibody component
EIVLTQSPGTLSLSPGERATLSCRASQSVDSTALAWYQQKPGQAPRLLIYAASSRATGIPDRFSGSGSGTDFTLTISRLEPEDFAVYYCQQDGEYPLTFGQGTKVEIKGGGGSGGGGSGGGSGGGGSEVQLLESGGGLVQPGGSLRLSCAASGFTFSDDYMSWVRQAPGKGLEWVSVISGSGGSTDYADSVKGRFTISRDNSKNTLYLQMNSLRAEDTAVYYCATGVPYCSTTRCPPYYYTMDVWGQGTTVTVSS

SEQ ID NO: 10 - DNA, 765 bp, synthetic construct
  misc_feature 1..765: note = Description of sequence: antibody component
  variation 762: note = n is a, c, g, or t
  source 1..765: mol_type = other DNA
gaaattgtgttgacgcagtctccaggcaccctgtctttgtctccaggggaacgtgccaccctctcctgccgtgccagtcagagtgttgacagcaccgccttagcctggtatcagcagaaacctggccaggctccccgactcctcatctatgccgcatctagccgtgccactggtatcccagaccgtttcagtggcagtgggtctgggacagacttcactctcaccatcagcagactggagcctgaagattttgcagtgtattactgtcagcaggacggcgagtatcctctgacgttcggccaaggtaccaaggtggaaatcaaaggtggtggtggttcaggtggtggtggttctggcggcggctccggtggtggtggatccgaggtgcagctgttggagtctgggggaggcttggtacagcctggggggtccctgcgactctcctgtgcagcctctggattcacctttagcgacgactatatgagctgggtccgccaggctccagggaaggggctggagtgggtgtcagtgattagcggtagcggtggtagcacagactacgcagactccgtgaagggccggttcaccatctcccgtgacaattccaagaacacgctgtatctgcaaatgaacagcctgcgtgccgaggacacggctgtgtattactgtgcgacaggggtcccatattgtagtactaccaggtgccccccatactactacactatggacgtctggggccaagggaccacggtcactgtctcntca

SEQ ID NO: 11 - protein, 8 aa, synthetic construct
  REGION 1..8: note = Description of sequence: antibody component
GFTFSSDG

SEQ ID NO: 12 - protein, 16 aa, synthetic construct
  REGION 1..16: note = Description of sequence: antibody component
ARETVWDPLSLGAFDI

SEQ ID NO: 13 - protein, 7 aa, synthetic construct
  REGION 1..7: note = Description of sequence: antibody component
QSVQASS

SEQ ID NO: 14 - protein, 9 aa, synthetic construct
  REGION 1..9: note = Description of sequence: antibody component
QQYGSSPIT

SEQ ID NO: 15 - protein, 123 aa, synthetic construct
  REGION 1..123: note = Description of sequence: antibody component
EVQLLESGGGLVQPGGSLRLSCAASGFTFSSDGMSWVRQAPGKGLEWVSAISGSGGSTNYADSVKGRFTISRDNSKNTLYLQMNSLRAEDTAVYYCARETVWDPLSLGAFDIWGQGTMVTVSS

SEQ ID NO: 16 - protein, 108 aa, synthetic construct
  REGION 1..108: note = Description of sequence: antibody component
EIVLTQSPGTLSLSPGERATLSCRASQSVQASSLAWYQQKPGQAPRLLIYAASSRATGIPDRFSGSGSGTDFTLTISRLEPEDFAVYYCQQYGSSPITFGQGTKVEIK

SEQ ID NO: 17 - protein, 250 aa, synthetic construct
  REGION 1..250: note = Description of sequence: antibody component
EIVLTQSPGTLSLSPGERATLSCRASQSVQASSLAWYQQKPGQAPRLLIYAASSRATGIPDRFSGSGSGTDFTLTISRLEPEDFAVYYCQQYGSSPITFGQGTKVEIKGGGGSGGGGSGGGSGGGGSEVQLLESGGGLVQPGGSLRLSCAASGFTFSSDGMSWVRQAPGKGLEWVSAISGSGGSTNYADSVKGRFTISRDNSKNTLYLQMNSLRAEDTAVYYCARETVWDPLSLGAFDIWGQGTMVTVSS

SEQ ID NO: 18 - DNA, 750 bp, synthetic construct
  misc_feature 1..750: note = Description of sequence: antibody component
  source 1..750: mol_type = other DNA
gaaattgtgttgacgcagtctccaggcaccctgtctttgtctccaggggaacgtgccaccctctcctgccgtgccagtcagagtgttcaggccagcagcttagcctggtatcagcagaaacctggccaggctccccgactcctcatctatgccgcatctagccgtgccactggtatcccagaccgtttcagtggcagtgggtctgggacagacttcactctcaccatcagcagactggagcctgaagattttgcagtgtattactgtcagcagtatggcagcagccctatcacgttcggccaaggtaccaaggtggaaatcaaaggtggtggtggttcaggtggtggtggttctggcggcggctccggtggtggtggatccgaggtgcagctgttggagtctgggggaggcttggtacagcctggggggtccctgcgactctcctgtgcagcctctggattcacctttagcagcgacggcatgagctgggtccgccaggctccagggaaggggctggagtgggtgtcagccattagcggtagcggtggtagcacaaattacgcagactccgtgaagggccggttcaccatctcccgtgacaattccaagaacacgctgtatctgcaaatgaacagcctgcgtgccgaggacacggccgtgtattactgtgcgagagagacggtgtgggatcccctatccctgggtgcttttgatatctggggccaagggacaatggtcaccgtctcttca

SEQ ID NO: 19 - protein, 8 aa, synthetic construct
  REGION 1..8: note = Description of sequence: antibody component
GFTFTDYY

SEQ ID NO: 20 - protein, 12 aa, synthetic construct
  REGION 1..12: note = Description of sequence: antibody component
ARDWGGSIPLDI

SEQ ID NO: 21 - protein, 7 aa, synthetic construct
  REGION 1..7: note = Description of sequence: antibody component
QSVSHSY

SEQ ID NO: 22 - protein, 9 aa, synthetic construct
  REGION 1..9: note = Description of sequence: antibody component
QQYSYSPFT

SEQ ID NO: 23 - protein, 119 aa, synthetic construct
  REGION 1..119: note = Description of sequence: antibody component
EVQLLESGGGLVQPGGSLRLSCAASGFTFTDYYMSWVRQAPGKGLEWVSDISGSGGSTYYADSVKGRFTISRDNSKNTLYLQMNSLRAEDTAVYYCARDWGGSIPLDIWGQGTMVTVSS

SEQ ID NO: 24 - protein, 108 aa, synthetic construct
  REGION 1..108: note = Description of sequence: antibody component
EIVLTQSPGTLSLSPGERATLSCRASQSVSHSYLAWYQQKPGQAPRLLIYAASSRATGIPDRFSGSGSGTDFTLTISRLEPEDFAVYYCQQYSYSPFTFGQGTKVEIK

SEQ ID NO: 25 - protein, 246 aa, synthetic construct
  REGION 1..246: note = Description of sequence: antibody component
EIVLTQSPGTLSLSPGERATLSCRASQSVSHSYLAWYQQKPGQAPRLLIYAASSRATGIPDRFSGSGSGTDFTLTISRLEPEDFAVYYCQQYSYSPFTFGQGTKVEIKGGGGSGGGGSGGGSGGGGSEVQLLESGGGLVQPGGSLRLSCAASGFTFTDYYMSWVRQAPGKGLEWVSDISGSGGSTYYADSVKGRFTISRDNSKNTLYLQMNSLRAEDTAVYYCARDWGGSIPLDIWGQGTMVTVSS

SEQ ID NO: 26 - DNA, 711 bp, synthetic construct
  misc_feature 1..711: note = Description of sequence: antibody component
  source 1..711: mol_type = other DNA
gaaattgtgttgacgcagtctccaggcaccctgtctttgtctccaggggaacgtgccaccctctcctgccgtgccagtcagagtgttagccacagctatttagcctggtatcagcagaaacctggccaggctccccgactcctcatctatgccgcatctagccgtgccactggtatcccagaccgtttcagtggcagtgggtctgggacagacttcactctcaccatcagcagactggagcctgaagattttgcagtgtattactgtcagcagtatagctatagcccttttacgttcggccaaggtaccaaggtggaaatcaaaggtggtggtggttcaggtggtggtggttctgaggtgcagctgttggagtctgggggaggcttggtacagcctggggggtccctgcgactctcctgtgcagcctctggattcacctttaccgactattatatgagctgggtccgccaggctccagggaaggggctggagtgggtgtcagacattagcggtagtggtggtagcacatactacgcagactccgtgaagggccggttcaccatctcccgtgacaattccaagaacacgctgtatctgcaaatgaacagcctgcgtgccgaggacacggccgtgtattactgtgcgagggattgggggggttccatccccctagatatctggggccaagggacaatggtcaccgtctcttca

SEQ ID NO: 27 - protein, 8 aa, synthetic construct
  REGION 1..8: note = Description of sequence: antibody component
ISGRGGQT

SEQ ID NO: 28 - protein, 16 aa, synthetic construct
  REGION 1..16: note = Description of sequence: antibody component
ARDSYLTIWSGEGFDY

SEQ ID NO: 29 - protein, 7 aa, synthetic construct
  REGION 1..7: note = Description of sequence: antibody component
QSVDRSY

SEQ ID NO: 30 - protein, 9 aa, synthetic construct
  REGION 1..9: note = Description of sequence: antibody component
QQDSYSPIT

SEQ ID NO: 31 - protein, 123 aa, synthetic construct
  REGION 1..123: note = Description of sequence: antibody component
EVQLLESGGGLVQPGGSLRLSCAASGFTFTDYYMSWVRQAPGKGLEWVSRISGRGGQTDYADSVKGRFTISRDNSKNTLYLQMNSLRAEDTAVYYCARDSYLTIWSGEGFDYWGQGTLVTVSS

SEQ ID NO: 32 - protein, 108 aa, synthetic construct
  REGION 1..108: note = Description of sequence: antibody component
EIVLTQSPGTLSLSPGERATLSCRASQSVDRSYLAWYQQKPGQAPRLLIYGASSRATGIPDRFSGSGSGTDFTLTISRLEPEDFAVYYCQQDSYSPITFGQGTKVEIK

SEQ ID NO: 33 - protein, 250 aa, synthetic construct
  REGION 1..250: note = Description of sequence: antibody component
EIVLTQSPGTLSLSPGERATLSCRASQSVDRSYLAWYQQKPGQAPRLLIYGASSRATGIPDRFSGSGSGTDFTLTISRLEPEDFAVYYCQQDSYSPITFGQGTKVEIKGGGGSGGGGSGGGSGGGGSEVQLLESGGGLVQPGGSLRLSCAASGFTFTDYYMSWVRQAPGKGLEWVSRISGRGGQTDYADSVKGRFTISRDNSKNTLYLQMNSLRAEDTAVYYCARDSYLTIWSGEGFDYWGQGTLVTVSS

SEQ ID NO: 34 - DNA, 750 bp, synthetic construct
  misc_feature 1..750: note = Description of sequence: antibody component
  source 1..750: mol_type = other DNA
gaaattgtgttgacgcagtctccaggcaccctgtctttgtctccaggggaacgtgccaccctctcctgccgtgccagtcagagtgttgaccgcagctatttagcctggtatcagcagaaacctggccaggctccccgactcctcatctatggcgcatctagccgtgccactggtatcccagaccgtttcagtggcagtgggtctgggacagacttcactctcaccatcagcagactggagcctgaagattttgcagtgtattactgtcagcaggacagctatagccctatcacgttcggccaaggtaccaaggtggaaatcaaaggtggtggtggttcaggtggtggtggttctggcggcggctccggtggtggtggatccgaggtgcagctgttggagtctgggggaggcttggtacagcctggggggtccctgcgactctcctgtgcagcctctggattcacctttaccgactattatatgagctgggtccgccaggctccagggaaggggctggagtgggtgtcacgcattagcggtcgcggtggtcagacagactacgcagactccgtgaagggccggttcaccatctcccgtgacaattccaagaacacgctgtatctgcaaatgaacagcctgcgtgccgaggacacggctgtgtattactgtgcgagagattcttacctcacaatatggtccggggaggggtttgactactggggccagggaaccctggtcaccgtctcctca

SEQ ID NO: 35 - protein, 8 aa, synthetic construct
  REGION 1..8: note = Description of sequence: antibody component
GFTFTSYA

SEQ ID NO: 36 - protein, 10 aa, synthetic construct
  REGION 1..10: note = Description of sequence: antibody component
ISGSGYGGST

SEQ ID NO: 37 - protein, 16 aa, synthetic construct
  REGION 1..16: note = Description of sequence: antibody component
VKDKSHTRVEADAFDI

SEQ ID NO: 38 - protein, 12 aa, synthetic construct
  REGION 1..12: note = Description of sequence: antibody component
QSVLSSNNNENN

SEQ ID NO: 39 - skipped

SEQ ID NO: 40 - protein, 9 aa, synthetic construct
  REGION 1..9: note = Description of sequence: antibody component
QQGTSSPIT

SEQ ID NO: 41 - protein, 125 aa, synthetic construct
  REGION 1..125: note = Description of sequence: antibody component
EVQLLESGGGLVQPGGSLRLSCAASGFTFTSYAMSWVRQAPGKGLEWVSRISGSGYGGSTYYADSVKGRFTISRDNSKNTLYLQMNSLRAEDTAVYYCVKDKSHTRVEADAFDIWGQGTMVTVSS

SEQ ID NO: 42 - protein, 113 aa, synthetic construct
  REGION 1..113: note = Description of sequence: antibody component
DIVMTQSPDSLAVSLGERATINCKSSQSVLSSNNNENNLAWYQQKPGQPPKLLIYDASTRESGVPDRFSGSGSGTDFTLTISSLQAEDVAVYYCQQGTSSPITFGQGTKVEIK

SEQ ID NO: 43 - protein, 257 aa, synthetic construct
  REGION 1..257: note = Description of sequence: antibody component
DIVMTQSPDSLAVSLGERATINCKSSQSVLSSNNNENNLAWYQQKPGQPPKLLIYDASTRESGVPDRFSGSGSGTDFTLTISSLQAEDVAVYYCQQGTSSPITFGQGTKVEIKGGGGSGGGGSGGGSGGGGSEVQLLESGGGLVQPGGSLRLSCAASGFTFTSYAMSWVRQAPGKGLEWVSRISGSGYGGSTYYADSVKGRFTISRDNSKNTLYLQMNSLRAEDTAVYYCVKDKSHTRVEADAFDIWGQGTMVTVSS

SEQ ID NO: 44 - DNA, 771 bp, synthetic construct
  misc_feature 1..771: note = Description of sequence: antibody component
  source 1..771: mol_type = other DNA
gacatcgtgatgacccagtctccagactccctggctgtgtctctgggcgagcgtgccaccatcaactgcaagtccagccagagtgttttaagtagcaataacaatgagaacaatttagcttggtatcagcagaaaccaggacagcctcctaagctgctcatttacgacgcatctacccgggaatccggggtccctgaccgattcagtggcagcgggtctgggacagatttcactctcaccatcagcagcctgcaggctgaagatgtggcagtttattactgtcagcaaggcaccagcagccctatcacgttcggccaaggtaccaaggtggaaatcaaaggtggtggtggttcaggtggtggtggttctggcggcggctccggtggtggtggatccgaggtgcagctgttggagtctgggggaggcttggtacagcctggggggtccctgcgactctcctgtgcagcctctggattcacctttaccagctatgccatgagctgggtccgccaggctccagggaaggggctggagtgggtgtcacgcattagcggtagcggttatggtggtagcacatattacgcagactccgtgaagggccggttcaccatctcccgtgacaattccaagaacacgctgtatctgcaaatgaacagcctgcgtgccgaggacacggctgtgtattactgtgtaaaagataagtcgcatactcgggttgaggcggatgcttttgatatctggggccaagggacaatggtcaccgtctcttca

SEQ ID NO: 45 - protein, 8 aa, synthetic construct
  REGION 1..8: note = Description of sequence: antibody component
GFTFSSYG

SEQ ID NO: 46 - protein, 8 aa, synthetic construct
  REGION 1..8: note = Description of sequence: antibody component
ISGYGSST

SEQ ID NO: 47 - protein, 15 aa, synthetic construct
  REGION 1..15: note = Description of sequence: antibody component
AKDRYSLSYYYGMDV

SEQ ID NO: 48 - protein, 12 aa, synthetic construct
  REGION 1..12: note = Description of sequence: antibody component
QSVLSSSNNYNR

SEQ ID NO: 49 - protein, 9 aa, synthetic construct
  REGION 1..9: note = Description of sequence: antibody component
QQYDSRPIT

SEQ ID NO: 50 - protein, 122 aa, synthetic construct
  REGION 1..122: note = Description of sequence: antibody component
EVQLLESGGGLVQPGGSLRLSCAASGFTFSSYGMSWVRQAPGKGLEWVSDISGYGSSTYYADSVKGRFTISRDNSKNTLYLQMNSLRAEDTAVYYCAKDRYSLSYYYGMDVWGQGTTVTVSS

SEQ ID NO: 51 - protein, 113 aa, synthetic construct
  REGION 1..113: note = Description of sequence: antibody component
DIVMTQSPDSLAVSLGERATINCKSSQSVLSSSNNYNRLAWYQQKPGQPPKLLIYAASTRESGVPDRFSGSGSGTDFTLTISSLQAEDVAVYYCQQYDSRPITFGQGTKVEIK

SEQ ID NO: 52 - protein, 254 aa, synthetic construct
  REGION 1..254: note = Description of sequence: antibody component
DIVMTQSPDSLAVSLGERATINCKSSQSVLSSSNNYNRLAWYQQKPGQPPKLLIYAASTRESGVPDRFSGSGSGTDFTLTISSLQAEDVAVYYCQQYDSRPITFGQGTKVEIKGGGGSGGGGSGGGSGGGGSEVQLLESGGGLVQPGGSLRLSCAASGFTFSSYGMSWVRQAPGKGLEWVSDISGYGSSTYYADSVKGRFTISRDNSKNTLYLQMNSLRAEDTAVYYCAKDRYSLSYYYGMDVWGQGTTVTVSS

SEQ ID NO: 53 - DNA, 762 bp, synthetic construct
  misc_feature 1..762: note = Description of sequence: antibody component
  source 1..762: mol_type = other DNA
gacatcgtgatgacccagtctccagactccctggctgtgtctctgggcgagcgtgccaccatcaactgcaagtccagccagagtgttttaagcagcagcaacaattataaccgcttagcttggtatcagcagaaaccaggacagcctcctaagctgctcatttacgccgcatctacccgggaatccggggtccctgaccgattcagtggcagcgggtctgggacagatttcactctcaccatcagcagcctgcaggctgaagatgtggcagtttattactgtcagcaatatgacagccgccctatcacgttcggccaaggtaccaaggtggaaatcaaaggtggtggtggttcaggtggtggtggttctggcggcggctccggtggtggtggatccgaggtgcagctgttggagtctgggggaggcttggtacagcctggggggtccctgcgactctcctgtgcagcctctggattcacctttagcagctatggcatgagctgggtccgccaggctccagggaaggggctggagtgggtgtcagacattagcggttatggtagcagcacatattacgcagactccgtgaagggccggttcaccatctcccgtgacaattccaagaacacgctgtatctgcaaatgaacagcctgcgtgccgaggacacggctgtgtattactgtgcaaaagaccggtatagcctttcctactactacggtatggacgtctggggccaagggaccacggtcaccgtctcctca

SEQ ID NO: 54 - protein, 8 aa, synthetic construct
  REGION 1..8: note = Description of sequence: antibody component
GFTFTSSA

SEQ ID NO: 55 - protein, 8 aa, synthetic construct
  REGION 1..8: note = Description of sequence: antibody component
IYGGGGST

SEQ ID NO: 56 - protein, 14 aa, synthetic construct
  REGION 1..14: note = Description of sequence: antibody component
ARAVWTSNGYYFDT

SEQ ID NO: 57 - protein, 12 aa, synthetic construct
  REGION 1..12: note = Description of sequence: antibody component
QSVLYSSNNKNN

SEQ ID NO: 58 - protein, 9 aa, synthetic construct
  REGION 1..9: note = Description of sequence: antibody component
QQGYSEPIT

SEQ ID NO: 59 - protein, 121 aa, synthetic construct
  REGION 1..121: note = Description of sequence: antibody component
EVQLLESGGGLVQPGGSLRLSCAASGFTFTSSAMSWVRQAPGKGLEWVSDIYGGGGSTSYADSVKGRFTISRDNSKNTLYLQMNSLRAEDTAVYYCARAVWTSNGYYFDTWGQGTLVTVSS

SEQ ID NO: 60 - protein, 113 aa, synthetic construct
  REGION 1..113: note = Description of sequence: antibody component
DIVMTQSPDSLAVSLGERATINCKSSQSVLYSSNNKNNLAWYQQKPGQPPKLLIYAASTRESGVPDRFSGSGSGTDFTLTISSLQAEDVAVYYCQQGYSEPITFGQGTKVEIK

SEQ ID NO: 61 - protein, 253 aa, synthetic construct
  REGION 1..253: note = Description of sequence: antibody component
DIVMTQSPDSLAVSLGERATINCKSSQSVLYSSNNKNNLAWYQQKPGQPPKLLIYAASTRESGVPDRFSGSGSGTDFTLTISSLQAEDVAVYYCQQGYSEPITFGQGTKVEIKGGGGSGGGGSGGGSGGGGSEVQLLESGGGLVQPGGSLRLSCAASGFTFTSSAMSWVRQAPGKGLEWVSDIYGGGGSTSYADSVKGRFTISRDNSKNTLYLQMNSLRAEDTAVYYCARAVWTSNGYYFDTWGQGTLVTVSS

SEQ ID NO: 62 - DNA, 759 bp, synthetic construct
  misc_feature 1..759: note = Description of sequence: antibody component
  source 1..759: mol_type = other DNA
gacatcgtgatgacccagtctccagactccctggctgtgtctctgggcgagcgtgccaccatcaactgcaagtccagccagagtgttttatatagcagcaacaataaaaacaatttagcttggtatcagcagaaaccaggacagcctcctaagctgctcatttacgccgcatctacccgggaatccggggtccctgaccgattcagtggcagcgggtctgggacagatttcactctcaccatcagcagcctgcaggctgaagatgtggcagtttattactgtcagcaaggctatagcgaacctatcacgttcggccaaggtaccaaggtggaaatcaaaggtggtggtggttcaggtggtggtggttctggcggcggctccggtggtggtggatccgaggtgcagctgttggagtctgggggaggcttggtacagcctggggggtccctgcgactctcctgtgcagcctctggattcacctttaccagcagcgccatgagctgggtccgccaggctccagggaaggggctggagtgggtgtcagacatttatggtggcggtggtagcacaagctacgcagactccgtgaagggccggttcaccatctcccgtgacaattccaagaacacgctgtatctgcaaatgaacagcctgcgtgccgaggacacggctgtgtattactgtgcaagagccgtctggacgagtaatggttattacttcgacacctggggccagggaaccctggtcaccgtctcctca

SEQ ID NO: 63 - protein, 8 aa, synthetic construct
  REGION 1..8: note = Description of sequence: antibody component
GFTFSDYA

SEQ ID NO: 64 - protein, 8 aa, synthetic construct
  REGION 1..8: note = Description of sequence: antibody component
IQGGGGYT

SEQ ID NO: 65 - protein, 24 aa, synthetic construct
  REGION 1..24: note = Description of sequence: antibody component
AKDQLEHYDFWSGYLNYYYYGMDV

SEQ ID NO: 66 - protein, 7 aa, synthetic construct
  REGION 1..7: note = Description of sequence: antibody component
QSVSSSY

SEQ ID NO: 67 - skipped

SEQ ID NO: 68 - protein, 9 aa, synthetic construct
  REGION 1..9: note = Description of sequence: antibody component
QQYSRSPLT

SEQ ID NO: 69 - protein, 131 aa, synthetic construct
  REGION 1..131: note = Description of sequence: antibody component
EVQLLESGGGLVQPGGSLRLSCAASGFTFSDYAMSWVRQAPGKGLEWVSEIQGGGGYTNYADSVKGRFTISRDNSKNTLYLQMNSLRAEDTAVYYCAKDQLEHYDFWSGYLNYYYYGMDVWGQGTTVTVSS

SEQ ID NO: 70 - protein, 108 aa, synthetic construct
  REGION 1..108: note = Description of sequence: antibody component
EIVLTQSPGTLSLSPGERATLSCRASQSVSSSYLAWYQQKPGQAPRLLIYGASSRATGIPDRFSGSGSGTDFTLTISRLEPEDFAVYYCQQYSRSPLTFGQGTKVEIK

SEQ ID NO: 71 - protein, 258 aa, synthetic construct
  REGION 1..258: note = Description of sequence: antibody component
EIVLTQSPGTLSLSPGERATLSCRASQSVSSSYLAWYQQKPGQAPRLLIYGASSRATGIPDRFSGSGSGTDFTLTISRLEPEDFAVYYCQQYSRSPLTFGQGTKVEIKGGGGSGGGGSGGGSGGGGSEVQLLESGGGLVQPGGSLRLSCAASGFTFSDYAMSWVRQAPGKGLEWVSEIQGGGGYTNYADSVKGRFTISRDNSKNTLYLQMNSLRAEDTAVYYCAKDQLEHYDFWSGYLNYYYYGMDVWGQGTTVTVSS

SEQ ID NO: 72 - DNA, 774 bp, synthetic construct
  misc_feature 1..774: note = Description of sequence: antibody component
  source 1..774: mol_type = other DNA
gaaattgtgttgacgcagtctccaggcaccctgtctttgtctccaggggaacgtgccaccctctcctgccgtgccagtcagagtgttagcagcagctatttagcctggtatcagcagaaacctggccaggctccccgactcctcatctatggcgcatctagccgtgccactggtatcccagaccgtttcagtggcagtgggtctgggacagacttcactctcaccatcagcagactggagcctgaagattttgcagtgtattactgtcagcagtatagccgcagccctctgacgttcggccaaggtaccaaggtggaaatcaaaggtggtggtggttcaggtggtggtggttctggcggcggctccggtggtggtggatccgaggtgcagctgttggagtctgggggaggcttggtacagcctggggggtccctgcgactctcctgtgcagcctctggattcacctttagcgactatgccatgagctgggtccgccaggctccagggaaggggctggagtgggtgtcagagattcagggtggcggtggttatacaaattacgcagactccgtgaagggccggttcaccatctcccgtgacaattccaagaacacgctgtatctgcaaatgaacagcctgcgtgccgaggacacggccgtgtattactgtgcgaaagatcaattagagcattacgatttttggagtggttacctgaactactactactacggtatggacgtctggggccaagggaccacggtcaccgtctcctca

SEQ ID NO: 73 - protein, 8 aa, synthetic construct
  REGION 1..8: note = Description of sequence: antibody component
GFTFSSYA

SEQ ID NO: 74 - protein, 8 aa, synthetic construct
  REGION 1..8: note = Description of sequence: antibody component
ISGSGGDT

SEQ ID NO: 75 - protein, 24 aa, synthetic construct
  REGION 1..24: note = Description of sequence: antibody component
ANRDTRLYYDFWSGYWNAPHAFDI

SEQ ID NO: 76 - protein, 7 aa, synthetic construct
  REGION 1..7: note = Description of sequence: antibody component
QSVSSTS

SEQ ID NO: 77 - protein, 9 aa, synthetic construct
  REGION 1..9: note = Description of sequence: antibody component
QQYSEYPLT

SEQ ID NO: 78 - protein, 131 aa, synthetic construct
  REGION 1..131: note = Description of sequence: antibody component
EVQLLESGGGLVQPGGSLRLSCAASGFTFSSYAMSWVRQAPGKGLEWVSEISGSGGDTKYADSVKGRFTISRDNSKNTLYLQMNSLRAEDTAVYYCANRDTRLYYDFWSGYWNAPHAFDIWGQGTMVTVSS

SEQ ID NO: 79 - protein, 108 aa, synthetic construct
  REGION 1..108: note = Description of sequence: antibody component
EIVLTQSPGTLSLSPGERATLSCRASQSVSSTSLAWYQQKPGQAPRLLIYGASSRATGIPDRFSGSGSGTDFTLTISRLEPEDFAVYYCQQYSEYPLTFGQGTKVEIK

SEQ ID NO: 80 - protein, 258 aa, synthetic construct
  REGION 1..258: note = Description of sequence: antibody component
EIVLTQSPGTLSLSPGERATLSCRASQSVSSTSLAWYQQKPGQAPRLLIYGASSRATGIPDRFSGSGSGTDFTLTISRLEPEDFAVYYCQQYSEYPLTFGQGTKVEIKGGGGSGGGGSGGGSGGGGSEVQLLESGGGLVQPGGSLRLSCAASGFTFSSYAMSWVRQAPGKGLEWVSEISGSGGDTKYADSVKGRFTISRDNSKNTLYLQMNSLRAEDTAVYYCANRDTRLYYDFWSGYWNAPHAFDIWGQGTMVTVSS

SEQ ID NO: 81 - DNA, 775 bp, synthetic construct
  misc_feature 1..775: note = Description of sequence: antibody component
  source 1..775: mol_type = other DNA
gaaattgtgttgacgcagtctccaggcaccctgtctttgtctccaggggaacgtgccaccctctcctgccgtgccagtcagagtgttagcagcaccagcttagcctggtatcagcagaaacctggccaggctccccgactcctcatctatggcgcatctagccgtgccactggtatcccagaccgtttcagtggcagtgggtctgggacagacttcactctcaccatcagcagactggagcctgaagattttgcagtgtattactgtcagcagtatagcgagtatcctctgacgttcggccaaggtaccaaggtggaaatcaaaggtggtggtggttcaggtggtggtggttctggcggcggctccggtggtggtggatccgaggtgcagctgttggagtctgggggaggcttggtacagcctggggggtccctgcgactctcctgtgcagcctctggattcacctttagcagctatgccatgagctgggtccgccaggctccagggaaggggctggagtgggtgtcagagattagcggtagcggtggtgacacaaaatacgcagactccgtgaagggccggttcaccatctcccgtgacaattccaagaacacgctgtatctgcaaatgaacagcctgcgtgccgaggacacggccgtgtattactgtgcgaaccgcgacacgcgcctttattacgatttttggagtggttattggaatgccccccatgcttttgatatctggggccaagggacaatggtcaccgtctcttcag

SEQ ID NO: 82 - protein, 8 aa, synthetic construct
  REGION 1..8: note = Description of sequence: antibody component
ISGSGGQT

SEQ ID NO: 83 - protein, 16 aa, synthetic construct
  REGION 1..16: note = Description of sequence: antibody component
ARDRTMGSYYYYGMDV

SEQ ID NO: 84 - protein, 7 aa, synthetic construct
  REGION 1..7: note = Description of sequence: antibody component
QSVSSNS

SEQ ID NO: 85 - protein, 9 aa, synthetic construct
  REGION 1..9: note = Description of sequence: antibody component
QQYEQSPIT

SEQ ID NO: 86 - protein, 123 aa, synthetic construct
  REGION 1..123: note = Description of sequence: antibody component
EVQLLESGGGLVQPGGSLRLSCAASGFTFSSYGMSWVRQAPGKGLEWVSAISGSGGQTNYADSVKGRFTISRDNSKNTLYLQMNSLRAEDTAVYYCARDRTMGSYYYYGMDVWGQGTTVTVSS

SEQ ID NO: 87 - protein, 108 aa, synthetic construct
  REGION 1..108: note = Description of sequence: antibody component
EIVLTQSPGTLSLSPGERATLSCRASQSVSSNSLAWYQQKPGQAPRLLIYGASSRATGIPDRFSGSGSGTDFTLTISRLEPEDFAVYYCQQYEQSPITFGQGTKVEIK

SEQ ID NO: 88 - protein, 250 aa, synthetic construct
  REGION 1..250: note = Description of sequence: antibody component
EIVLTQSPGTLSLSPGERATLSCRASQSVSSNSLAWYQQKPGQAPRLLIYGASSRATGIPDRFSGSGSGTDFTLTISRLEPEDFAVYYCQQYEQSPITFGQGTKVEIKGGGGSGGGGSGGGSGGGGSEVQLLESGGGLVQPGGSLRLSCAASGFTFSSYGMSWVRQAPGKGLEWVSAISGSGGQTNYADSVKGRFTISRDNSKNTLYLQMNSLRAEDTAVYYCARDRTMGSYYYYGMDVWGQGTTVTVSS

SEQ ID NO: 89 - DNA, 750 bp, synthetic construct
  misc_feature 1..750: note = Description of sequence: antibody component
  source 1..750: mol_type = other DNA
gaaattgtgttgacgcagtctccaggcaccctgtctttgtctccaggggaacgtgccaccctctcctgccgtgccagtcagagtgttagcagcaatagcttagcctggtatcagcagaaacctggccaggctccccgactcctcatctatggcgcatctagccgtgccactggtatcccagaccgtttcagtggcagtgggtctgggacagacttcactctcaccatcagcagactggagcctgaagattttgcagtgtattactgtcagcagtatgagcagagccctatcacgttcggccaaggtaccaaggtggaaatcaaaggtggtggtggttcaggtggtggtggttctggcggcggctccggtggtggtggatccgaggtgcagctgttggagtctgggggaggcttggtacagcctggggggtccctgcgactctcctgtgcagcctctggattcacctttagcagctatggcatgagctgggtccgccaggctccagggaaggggctggagtgggtgtcagccattagcggtagcggtggtcagacaaattacgcagactccgtgaagggccggttcaccatctcccgtgacaattccaagaacacgctgtatctgcaaatgaacagcctgcgtgccgaggacacggctgtgtattactgtgcgagagatagaactatggggagctactactactacggtatggacgtctggggccaagggaccacggtcaccgtctcctca

SEQ ID NO: 90 - protein, 8 aa, synthetic construct
  REGION 1..8: note = Description of sequence: antibody component
GFTFSDYY

SEQ ID NO: 91 - protein, 8 aa, synthetic construct
  REGION 1..8: note = Description of sequence: antibody component
ISGSGSYT

SEQ ID NO: 92 - protein, 8 aa, synthetic construct
  REGION 1..8: note = Description of sequence: antibody component
AQGWAFES

SEQ ID NO: 93 - protein, 7 aa, synthetic construct
  REGION 1..7: note = Description of sequence: antibody component
QSVSSSY

SEQ ID NO: 94 - protein, 9 aa, synthetic construct
  REGION 1..9: note = Description of sequence: antibody component
QQYSRSPLT

SEQ ID NO: 95 - protein, 115 aa, synthetic construct
  REGION 1..115: note = Description of sequence: antibody component
EVQLLESGGGLVQPGGSLRLSCAASGFTFSDYYMSWVRQAPGKGLEWVSDISGSGSYTRYADSVKGRFTISRDNSKNTLYLQMNSLRAEDTAVYYCAQGWAFESWGQGTLVTVSS

SEQ ID NO: 96 - protein, 108 aa, synthetic construct; identical to SEQ ID NO: 70
  REGION 1..108: note = Description of sequence: antibody component

SEQ ID NO: 97 - protein, 242 aa, synthetic construct
  REGION 1..242: note = Description of sequence: antibody component
EIVLTQSPGTLSLSPGERATLSCRASQSVSSSYLAWYQQKPGQAPRLLIYGASSRATGIPDRFSGSGSGTDFTLTISRLEPEDFAVYYCQQYSRSPLTFGQGTKVEIKGGGGSGGGGSGGGSGGGGSEVQLLESGGGLVQPGGSLRLSCAASGFTFSDYYMSWVRQAPGKGLEWVSDISGSGSYTRYADSVKGRFTISRDNSKNTLYLQMNSLRAEDTAVYYCAQGWAFESWGQGTLVTVSS

SEQ ID NO: 98 - DNA, 727 bp, synthetic construct
  misc_feature 1..727: note = Description of sequence: antibody component
  source 1..727: mol_type = other DNA
gaaattgtgttgacgcagtctccaggcaccctgtctttgtctccaggggaacgtgccaccctctcctgccgtgccagtcagagtgttagcagcagctatttagcctggtatcagcagaaacctggccaggctccccgactcctcatctatggcgcatctagccgtgccactggtatcccagaccgtttcagtggcagtgggtctgggacagacttcactctcaccatcagcagactggagcctgaagattttgcagtgtattactgtcagcagtatagccgcagccctctgacgttcggccaaggtaccaaggtggaaatcaaaggtggtggtggttcaggtggtggtggttctggcggcggctccggtggtggtggatccgaggtgcagctgttggagtctgggggaggcttggtacagcctggggggtccctgcgactctcctgtgcagcctctggattcacctttagcgactattatatgagctgggtccgccaggctccagggaaggggctggagtgggtgtcagacattagcggtagcggtagctatacacgctacgcagactccgtgaagggccggttcaccatctcccgtgacaattccaagaacacgctgtatctgcaaatgaacagcctgcgtgccgaggacacggctgtgtattactgtgcacaaggctgggcttttgagtcctggggccagggaaccctggtcaccgtctcctcag

SEQ ID NO: 99 - protein, 14 aa, synthetic construct
  REGION 1..14: note = Description of sequence: antibody component
AKDIFSYLAEGMDV

SEQ ID NO: 100 - protein, 9 aa, synthetic construct
  REGION 1..9: note = Description of sequence: antibody component
QQYYEYPYT

SEQ ID NO: 101 - protein, 121 aa, synthetic construct
  REGION 1..121: note = Description of sequence: antibody component
EVQLLESGGGLVQPGGSLRLSCAASGFTFSSYGMSWVRQAPGKGLEWVSRISGYGSSTNYADSVKGRFTISRDNSKNTLYLQMNSLRAEDTAVYYCAKDIFSYLAEGMDVWGQGTTVTVSS

SEQ ID NO: 102 - protein, 108 aa, synthetic construct
  REGION 1..108: note = Description of sequence: antibody component
EIVLTQSPGTLSLSPGERATLSCRASQSVSSSYLAWYQQKPGQAPRLLIYGASSRATGIPDRFSGSGSGTDFTLTISRLEPEDFAVYYCQQYYEYPYTFGQGTKVEIK

SEQ ID NO: 103 - protein, 248 aa, synthetic construct
  REGION 1..248: note = Description of sequence: antibody component
EIVLTQSPGTLSLSPGERATLSCRASQSVSSSYLAWYQQKPGQAPRLLIYGASSRATGIPDRFSGSGSGTDFTLTISRLEPEDFAVYYCQQYYEYPYTFGQGTKVEIKGGGGSGGGGSGGGSGGGGSEVQLLESGGGLVQPGGSLRLSCAASGFTFSSYGMSWVRQAPGKGLEWVSRISGYGSSTNYADSVKGRFTISRDNSKNTLYLQMNSLRAEDTAVYYCAKDIFSYLAEGMDVWGQGTTVTVSS

SEQ ID NO: 104 - DNA, 744 bp, synthetic construct
  misc_feature 1..744: note = Description of sequence: antibody component
  source 1..744: mol_type = other DNA
gaaattgtgttgacgcagtctccaggcaccctgtctttgtctccaggggaacgtgccaccctctcctgccgtgccagtcagagtgttagcagcagctatttagcctggtatcagcagaaacctggccaggctccccgactcctcatctatggcgcatctagccgtgccactggtatcccagaccgtttcagtggcagtgggtctgggacagacttcactctcaccatcagcagactggagcctgaagattttgcagtgtattactgtcagcagtattatgagtatccttatacgttcggccaaggtaccaaggtggaaatcaaaggtggtggtggttcaggtggtggtggttctggcggcggctccggtggtggtggatccgaggtgcagctgttggagtctgggggaggcttggtacagcctggggggtccctgcgactctcctgtgcagcctctggattcacctttagcagctatggcatgagctgggtccgccaggctccagggaaggggctggagtgggtgtcacgcattagcggttatggtagcagcacaaattacgcagactccgtgaagggccggttcaccatctcccgtgacaattccaagaacacgctgtatctgcaaatgaacagcctgcgtgccgaggacacggctgtgtattactgtgcaaaagatatcttctcttatttggcggagggtatggacgtctggggccaagggaccacggtcaccgtctcctca

SEQ ID NO: 105 - protein, 8 aa, synthetic construct
  REGION 1..8: note = Description of sequence: antibody component
QASYLAWY

SEQ ID NO: 106 - protein, 8 aa, synthetic construct
  REGION 1..8: note = Description of sequence: antibody component
ISGSGDYT

SEQ ID NO: 107 - protein, 18 aa, synthetic construct
  REGION 1..18: note = Description of sequence: antibody component
ARETRQWLGLYYYYGMDV

SEQ ID NO: 108 - protein, 125 aa, synthetic construct
  REGION 1..125: note = Description of sequence: antibody component
TQSPGTLSLSPGERATLSCRASQSVQASYLAWYQQKPGQAPGKGLEWVSAISGSGDYTDYADSVKGRFTISRDNSKNTLYLQMNSLRAEDTAVYYCARETRQWLGLYYYYGMDVWGQGTTVTVSS

SEQ ID NO: 109 - DNA, 375 bp, synthetic construct
  misc_feature 1..375: note = Description of sequence: antibody component
  source 1..375: mol_type = other DNA
acgcagtctccaggcaccctgtctttgtctccaggggaacgtgccaccctctcctgccgtgccagtcagagtgttcaggccagctatttagcctggtatcagcagaaacctggccaggctccagggaaggggctggagtgggtgtcagctattagtggtagcggtgactatacagactacgcagactccgtgaagggccggttcaccatctcccgtgacaattccaagaacacgctgtatctgcaaatgaacagcctgcgtgccgaggacacggctgtgtattactgtgcgagagagacgcggcagtggctgggcctctactactactacggtatggacgtctggggccaagggaccacggtcaccgtctcctca

SEQ ID NO: 110 - protein, 19 aa, synthetic construct
  REGION 1..19: note = Description of sequence: antibody component
GGGGSGGGGSGGGSGGGGS

SEQ ID NO: 111 - protein, 15 aa, synthetic construct
  REGION 1..15: note = Description of sequence: antibody component
GGGGSGGGGSGGGGS

SEQ ID NO: 112 - protein, 24 aa, synthetic construct
  REGION 1..24: note = Description of sequence: antibody component
GGGGSGGGGSGGGGSGGGSGGGGS

SEQ ID NO: 113 - protein, 29 aa, synthetic construct
  REGION 1..29: note = Description of sequence: antibody component
GGGGSGGGGSGGGGSGGGGSGGGSGGGGS

SEQ ID NO: 114 - protein, 5 aa, synthetic construct
  REGION 1..5: note = Description of sequence: antibody component
GGGGS

SEQ ID NO: 115 - protein, 10 aa, synthetic construct
  REGION 1..10: note = Description of sequence: antibody component
GGGGSGGGGS

SEQ ID NO: 116 - protein, 335 aa, synthetic construct
  REGION 1..335: note = Description of sequence: antibody component
MGHPPLLPLLLLLHTCVPASWGLRCMQCKTNGDCRVEECALGQDLCRTTIVRLWEEGEELELVEKSCTHSEKTNRTLSYRTGLKITSLTEVVCGLDLCNQGNSGRAVTYSRSRYLECISCGSSDMSCERGRHQSLQCRSPEEQCLDVVTHWIQEGEEGRPKDDRHLRGCGYLPGCPGSNGFHNNDTFHFLKCCNTTKCNEGPILELENLPQNGRQCYSCKGNSTHGCSSEETFLIDCRGPMNQCLVATGTHEPKNQSYMVRGCATASMCQHAHLGDAFSMNHIDVSCCTKSGCNHPDLDVQYRSGAAPQPGPAHLSLTITLLMTARLWGGTLLWT